European Patent Application EP 4 420 519 A1, published August 28, 2024. Title: Method for treating and/or preventing bed bug infestations. Applicant: Izinovation. The sequence listing filed with the application follows.

SEQUENCE LISTING (2 sequences)

SEQ ID NO: 1 - DNA, 561 bp, Metarhizium robertsii
  source 1..561: mol_type = genomic DNA
gtcgtaacaaggtctccgttggtgaaccagcggagggatcattaccgagttatccaactcccaacccctgtgaattatacctttaattgttgcttcggcgggacttcgcgcccgccggggacccaaaccttctgaattttttaataagtatcttctgagtggttaaaaaaatgaatcaaaactttcaacaacggatctcttggttctggcatcgatgaagaacgcagcgaaatgcgataagtaatgtgaattgcagaattcagtgaatcatcgaatctttgaacgcacattgcgcccgtcagtattctggcgggcatgcctgttcgagcgtcattacgcccctcaagtcccctgtggacttggtgttggggatcggcgaggctggttttccagcacagccgtcccttaaattaattggcggtctcgccgtggccctcctctgcgcagtagtaaaacactcgcaacaggagcccggcgcggtccactgccgtaaaaccccccaactttttatagttgacctcgaatcaggtaggactacccgctgaacttaagcatatcaat

SEQ ID NO: 2 - DNA, 853 bp, Metarhizium robertsii
  source 1..853: mol_type = genomic DNA
tggtatctccaaggatggccagacccgtgagcacgctctcctcgcctacaccctgggtgtcaagcagctcattgtcgccatcaacaagatggacaccaccaagtggtccgaggcccgttaccaggaaatcatcaaggagacttccaacttcatcaagaaggtcggctacaaccccaagaccgtcgccttcgtccccatctccggtttccacggtgacaacatgcttcaggcctccaccaactgcccctggtacaagggttgggagaaggagaccaaggctggcaagtccaccggcaagaccctcctcgaggccattgacgccattgagccccccaagcgtcccaccgacaagcccctccgtcttcccctccaggatgtgtacaagattggcggtattggaactgtccctgtcggccgtatcgagactggtgtcctcaagcccggtatggtcgttaccttcgctccctccaacgtcaccactgaagtcaagtccgtggaaatgcaccacgagcagcttaccgagggtgtccccggtgacaacgttggtttcaacgtgaagaacgtttccgtcaaggaaatccgccgtggtaacgttgctggtgactccaagaacgacccccccatgggtgccgcttccttcgatgcccaggtcatcgttctcaaccaccccggccaggtcggtgctggttacgctcccgtcctcgattgccacaccgcccacattgcctgcaagttctctgagatcaaggagaagattgaccgacgtaccggtaaggctgttgagtctgcccccaagttcatcaagtctggtgactctgccatcgtcaagatggttccctccaagcctatgtgc